European Patent Specification EP 3 957 319 B1, published December 4, 2024. Title: TREATMENT OF HEPATITIS DELTA VIRUS INFECTION WITH INTERFERON LAMBDA. Applicant: EIGER BIOPHARMACEUTICALS, INC. Application EP 21164362.2. The sequence listing filed with the application follows.

SEQUENCE LISTING (1 sequence)

SEQ ID NO: 1 - protein, 176 aa, Artificial Sequence
  source: /note="Description of Artificial Sequence: Synthetic polypeptide"
MKPTTTGKGCHIGRFKSLSPQELASFKKARDALEESLKLKNWSCSSPVFPGNWDLRLLQVRERPVALEAELALTLKVLEAAAGPALEDVLDQPLHTLHHILSQLQACIQPQPTAGPRPRGRLHHWLHRLQEAPKKESAGCLEASVTFNLFRLLTRDLKYVADGNLSLRTSTHPEST